European Patent Specification EP 3 555 077 B1, published April 19, 2023. Title: Compositions and Methods for Treating Cancer. Applicant: The Regents of the University of California Shokat, Kevan M. Gentile, Daniel Moss, Steven. Application To be assigned. The sequence listing filed with the application follows.

SEQUENCE LISTING (66 sequences)

SEQ ID NO: 1 - protein, 169 aa, Artificial sequence
  Synthetic polypeptide
MTEYKLVVVGAGGVGKSALTIQLIQNHFVDEYDPTIEDSYRKQVVIDGETCLLDILDTAGQEEYSAMRDQYMRTGEGFLCVFAINNTKSFEDIHHYREQIKRVKDSEDVPMVLVGNKCDLPSRTVDTKQAQDLARSYGIPFIETSAKTRQGVDDAFYTLVREIRKHKEK

SEQ ID NO: 2 - protein, 188 aa, Artificial sequence [sequence omitted]

SEQ ID NO: 3 - protein, 188 aa, Artificial sequence [sequence omitted]

SEQ ID NO: 4 - protein, 166 aa, Artificial sequence [sequence omitted]

SEQ ID NO: 5 - protein, 189 aa, Artificial sequence
  Synthetic polypeptide
MTEYKLVVVGAGGVGKSALTIQLIQNHFVDEYDPTIEDSYRKQVVIDGETCLLDILDTAGQEEYSAMRDQYMRTGEGFLCVFAINNTKSFEDIHQYREQIKRVKDSDDVPMVLVGNKCDLAARTVESRQAQDLARSYGIPYIETSAKTRQGVEDAFYTLVREIRQHKLRKLNPPDESGPGCMSCKCVLS

SEQ ID NO: 6 - protein, 189 aa, Artificial sequence; identical to SEQ ID NO: 5
  Synthetic polypeptide

SEQ ID NO: 7 - protein, 16 aa, Artificial Sequence
  Synthetic polypeptide
YKLVVVGAGGVGKSAL

SEQ ID NO: 8 - protein, 15 aa, Artificial Sequence
  Synthetic polypeptide
KLVVVGAGGVGKSAL

SEQ ID NO: 9 - protein, 13 aa, Artificial Sequence
  Synthetic polypeptide
VVVGAGGVGKSAL

SEQ ID NO: 10 - protein, 14 aa, Artificial Sequence
  Synthetic polypeptide
VVVGAGGVGKSALT

SEQ ID NO: 11 - protein, 9 aa, Artificial Sequence
  Synthetic polypeptide
LIQNHFVDE

SEQ ID NO: 12 - protein, 8 aa, Artificial Sequence
  Synthetic polypeptide
IQNHFVDE

SEQ ID NO: 13 - protein, 14 aa, Artificial Sequence
  Synthetic polypeptide
IQNHFVDEYDPTIE

SEQ ID NO: 14 - protein, 16 aa, Artificial Sequence
  Synthetic polypeptide
IQNHFVDEYDPTIEDS

SEQ ID NO: 15 - protein, 13 aa, Artificial Sequence
  Synthetic polypeptide
HFVDEYDPTIEDS

SEQ ID NO: 16 - protein, 11 aa, Artificial Sequence
  Synthetic polypeptide
VDEYDPTIEDS

SEQ ID NO: 17 - protein, 6 aa, Artificial Sequence
  Synthetic polypeptide
YDPTIE

SEQ ID NO: 18 - protein, 7 aa, Artificial Sequence
  Synthetic polypeptide
YDPTIED

SEQ ID NO: 19 - protein, 8 aa, Artificial Sequence
  Synthetic polypeptide
YDPTIEDS

SEQ ID NO: 20 - protein, 15 aa, Artificial Sequence
  Synthetic polypeptide
DSYRKQVVIDGETCL

SEQ ID NO: 21 - protein, 12 aa, Artificial Sequence
  Synthetic polypeptide
SYRKQVVIDGET

SEQ ID NO: 22 - protein, 14 aa, Artificial Sequence
  Synthetic polypeptide
SYRKQVVIDGETCL

SEQ ID NO: 23 - protein, 9 aa, Artificial Sequence
  Synthetic polypeptide
YRKQVVIDG

SEQ ID NO: 24 - protein, 11 aa, Artificial Sequence
  Synthetic polypeptide
YRKQVVIDGET

SEQ ID NO: 25 - protein, 13 aa, Artificial Sequence
  Synthetic polypeptide
YRKQVVIDGETCL

SEQ ID NO: 26 - protein, 12 aa, Artificial Sequence
  Synthetic polypeptide
RKQVVIDGETCL

SEQ ID NO: 27 - protein, 10 aa, Artificial Sequence
  Synthetic polypeptide
LDILDTAGQE

SEQ ID NO: 28 - protein, 11 aa, Artificial Sequence
  Synthetic polypeptide
LDILDTAGQEE

SEQ ID NO: 29 - protein, 12 aa, Artificial Sequence
  Synthetic polypeptide
LDILDTAGQEEY

SEQ ID NO: 30 - protein, 7 aa, Artificial Sequence
  Synthetic polypeptide
DTAGQEE

SEQ ID NO: 31 - protein, 8 aa, Artificial Sequence
  Synthetic polypeptide
DTAGQEEY

SEQ ID NO: 32 - protein, 10 aa, Artificial Sequence
  Synthetic polypeptide
DTAGQEEYSA

SEQ ID NO: 33 - protein, 11 aa, Artificial Sequence
  Synthetic polypeptide
DTAGQEEYSAM

SEQ ID NO: 34 - protein, 8 aa, Artificial Sequence
  Synthetic polypeptide
YSAMRDQY

SEQ ID NO: 35 - protein, 11 aa, Artificial Sequence
  Synthetic polypeptide
RDQYCRTGEGF

SEQ ID NO: 36 - protein, 12 aa, Artificial Sequence
  Synthetic polypeptide
RDQYCRTGEGFL

SEQ ID NO: 37 - protein, 7 aa, Artificial Sequence
  Synthetic polypeptide
CRTGEGF

SEQ ID NO: 38 - protein, 8 aa, Artificial Sequence
  Synthetic polypeptide
CRTGEGFL

SEQ ID NO: 39 - protein, 8 aa, Artificial Sequence
  Synthetic polypeptide
FAINNTKS

SEQ ID NO: 40 - protein, 9 aa, Artificial Sequence
  Synthetic polypeptide
FAINNTKSF

SEQ ID NO: 41 - protein, 10 aa, Artificial Sequence
  Synthetic polypeptide
FAINNTKSFE

SEQ ID NO: 42 - protein, 14 aa, Artificial Sequence
  Synthetic polypeptide
FAINNTKSFEDIHQ

SEQ ID NO: 43 - protein, 9 aa, Artificial Sequence
  Synthetic polypeptide
AINNTKSFE

SEQ ID NO: 44 - protein, 13 aa, Artificial Sequence
  Synthetic polypeptide
AINNTKSFEDIHQ

SEQ ID NO: 45 - protein, 6 aa, Artificial Sequence
  Synthetic polypeptide
FEDIHQ

SEQ ID NO: 46 - protein, 24 aa, Artificial Sequence
  Synthetic polypeptide
FEDIHQYREQIKRVKDSDDVPMVL

SEQ ID NO: 47 - protein, 23 aa, Artificial Sequence
  Synthetic polypeptide
EDIHQYREQIKRVKDSDDVPMVL

SEQ ID NO: 48 - protein, 22 aa, Artificial Sequence
  Synthetic polypeptide
DIHQYREQIKRVKDSDDVPMVL

SEQ ID NO: 49 - protein, 18 aa, Artificial Sequence
  Synthetic polypeptide
YREQIKRVKDSDDVPMVL

SEQ ID NO: 50 - protein, 17 aa, Artificial Sequence
  Synthetic polypeptide
REQIKRVKDSDDVPMVL

SEQ ID NO: 51 - protein, 15 aa, Artificial Sequence
  Synthetic polypeptide
QIKRVKDSDDVPMVL

SEQ ID NO: 52 - protein, 7 aa, Artificial Sequence
  Synthetic polypeptide
VGNKCDL

SEQ ID NO: 53 - protein, 12 aa, Artificial Sequence
  Synthetic polypeptide
AARTVESRQAQD

SEQ ID NO: 54 - protein, 13 aa, Artificial Sequence
  Synthetic polypeptide
AARTVESRQAQDL

SEQ ID NO: 55 - protein, 16 aa, Artificial Sequence
  Synthetic polypeptide
AARTVESRQAQDLARS

SEQ ID NO: 56 - protein, 7 aa, Artificial Sequence
  Synthetic polypeptide
SRQAQDL

SEQ ID NO: 57 - protein, 12 aa, Artificial Sequence
  Synthetic polypeptide
LARSYGIPYIET

SEQ ID NO: 58 - protein, 11 aa, Artificial Sequence
  Synthetic polypeptide
ARSYGIPYIET

SEQ ID NO: 59 - protein, 13 aa, Artificial Sequence
  Synthetic polypeptide
ARSYGIPYIETSA

SEQ ID NO: 60 - protein, 23 aa, Artificial Sequence
  Synthetic polypeptide
ARSYGIPYIETSAKTRQGVEDAF

SEQ ID NO: 61 - protein, 8 aa, Artificial Sequence
  Synthetic polypeptide
YGIPYIET

SEQ ID NO: 62 - protein, 9 aa, Artificial Sequence
  Synthetic polypeptide
SAKTRQGVE

SEQ ID NO: 63 - protein, 11 aa, Artificial Sequence
  Synthetic polypeptide
SAKTRQGVEDA

SEQ ID NO: 64 - protein, 12 aa, Artificial Sequence
  Synthetic polypeptide
SAKTRQGVEDAF

SEQ ID NO: 65 - protein, 10 aa, Artificial Sequence
  Synthetic polypeptide
YTLVREIRQH

SEQ ID NO: 66 - protein, 7 aa, Artificial Sequence
  Synthetic polypeptide
VREIRQH